European Patent Application EP 4 166 196 A1, published April 19, 2023. Title: ANTIBODIES BINDING CD24, PREPARATION AND USE THEREOF. Applicant: ImmuneOnco Biopharmaceuticals (Shanghai) Co., Ltd. The sequence listing filed with the application follows.

SEQUENCE LISTING (22 sequences)

SEQ ID NO: 1 - protein, 9 aa, Artificial Sequence
  HV-CDR-1 of IMM47C, IMM47 and IMM47H
GYSITSGYS

SEQ ID NO: 2 - protein, 7 aa, Artificial Sequence
  HV-CDR-2 of IMM47C, IMM47 and IMM47H
IHYSGST

SEQ ID NO: 3 - protein, 10 aa, Artificial Sequence
  HV-CDR-3 of IMM47C, IMM47 and IMM47H
ARGADYALDY

SEQ ID NO: 4 - protein, 12 aa, Artificial Sequence
  LV-CDR-1 of IMM47C, IMM47 and IMM47H
QSLLYSSNQKNY

SEQ ID NO: 5 - protein, 3 aa, Artificial Sequence
  LV-CDR-2 of IMM47C, IMM47 and IMM47H
WAS

SEQ ID NO: 6 - protein, 9 aa, Artificial Sequence
  LV-CDR-3 of IMM47C, IMM47 and IMM47H
QQNFIYPLT

SEQ ID NO: 7 - protein, 117 aa, Artificial Sequence
  IMM47C/IMM47's heavy chain variable region
DVQLQESGPDLVKPSQSLSLTCTVTGYSITSGYSWHWIRQFPGNKLEWMGYIHYSGSTKYNPSLKSRISITRDTSKNQFFLQLNSVTTEDTATYFCARGADYALDYWGQRTSVTVSS

SEQ ID NO: 8 - protein, 113 aa, Artificial Sequence
  IMM47C's light chain variable region
DIVMSQSPSSLAVSVGEKVTMSCKSSQSLLYSSNQKNYLAWYQQKPGHSPKLLIYWASTRESGVPDRFTGSGSGTDFTLTISSVKAEDLAVYYCQQNFIYPLTFGAGTKLELK

SEQ ID NO: 9 - protein, 113 aa, Artificial Sequence
  IMM47's light chain variable region
DIQMTQSPSSLSASVGDRVTITCKSSQSLLYSSNQKNYLAWYQQKPGKAPKLLIYWASTRESGVPSRFSGSGSGTDFTLTISSLQPEDFATYYCQQNFIYPLTFGGGTKVELK

SEQ ID NO: 10 - protein, 117 aa, Artificial Sequence
  IMM47H's heavy chain variable region
DVQLQESGPGLVKPSETLSLTCTVSGYSITSGYSWHWIRQPPGKGLEWIGYIHYSGSTKYNPSLKSRVTISVDTSKNQFSLKLSSVTAADTAVYYCARGADYALDYWGQRTSVTVSS

SEQ ID NO: 11 - protein, 113 aa, Artificial Sequence
  IMM47H's light chain variable region
DIVMTQSPDSLAVSLGERATINCKSSQSLLYSSNQKNYLAWYQQKPGQPPKLLIYWASTRESGVPDRFSGSGSGTDFTLTISSLQAEDVAVYYCQQNFIYPLTFGGGTKVELK

SEQ ID NO: 12 - protein, 330 aa, Artificial Sequence
  Heavy chain constant region
ASTKGPSVFPLAPSSKSTSGGTAALGCLVKDYFPEPVTVSWNSGALTSGVHTFPAVLQSSGLYSLSSVVTVPSSSLGTQTYICNVNHKPSNTKVDKRVEPKSCDKTHTCPPCPAPELLGGPSVFLFPPKPKDTLMISRTPEVTCVVVDVSHEDPEVKFNWYVDGVEVHNAKTKPREEQYNATYRVVSVLTVLHQDWLNGKEYKCKVSNKALPAPIAATISKAKGQPREPQVYTLPPSREEMTKNQVSLTCLVKGFYPSDIAVEWESNGQPENNYKTTPPVLDSDGSFFLYSKLTVDKSRWQQGNVFSCSVMHEALHNHYTQKSLSLSPGK

SEQ ID NO: 13 - protein, 107 aa, Artificial Sequence [sequence omitted]

SEQ ID NO: 14 - DNA, 1398 bp, Artificial Sequence
  IMM47C/IMM47's heavy chain
atgagagtgctgattcttttgtgcctgttcacagcctttcctggtatcctgtctgatgtgcagcttcaggagtcaggacctgacctggtgaaaccttctcagtcactttcactcacctgcactgtcactggctactccatcaccagtggttatagctggcactggatccggcagtttccaggaaacaaactggaatggatgggctacatacactatagtggtagcactaagtacaacccatctctcaaaagtcgaatctctatcactcgagacacatccaagaaccagttcttcctgcagttgaattctgtgactactgaggacacagccacatatttctgtgcaagaggcgcggactatgctttggactactggggtcaacgaacctcagtcaccgtctcctcagctagcaccaagggcccatcggtcttccccctggcaccctcctccaagagcacctctgggggcacagcggccctgggctgcctggtcaaggactacttccccgaaccggtgacggtgtcgtggaactcaggcgccctgaccagcggcgtgcacaccttcccggctgtcctacagtcctcaggactctactccctcagcagcgtggtgaccgtgccctccagcagcttgggcacccagacctacatctgcaacgtgaatcacaagcccagcaacaccaaggtggacaagagagttgagcccaaatcttgtgacaaaactcacacatgcccaccgtgcccagcacctgaactcctggggggaccgtcagtcttcctcttccccccaaaacccaaggacaccctcatgatctcccggacccctgaggtcacatgcgtggtggtggacgtgagccacgaagaccctgaggtcaagttcaactggtatgtggacggcgtggaggtgcataatgccaagacaaagccgcgggaggagcagtacaacgccacgtaccgtgtggtcagcgtcctcaccgtcctgcaccaagactggctgaatggcaaggagtacaagtgcaaggtctccaacaaagccctcccagcccccatcgccgcaaccatctccaaagccaaagggcagccccgagaaccacaggtgtacaccctgcccccatcccgggaggagatgaccaagaaccaagtcagcctgacctgcctggtcaaaggcttctatcccagcgacatcgccgtggagtgggagagcaatgggcagccggagaacaactacaagaccacgcctcccgtgctggactccgacggctccttcttcctctattccaagctcaccgtggacaagagcaggtggcagcaggggaacgtcttctcatgctccgtgatgcatgaggctctgcacaaccactacacgcagaagagcctctccctgtctccgggcaaatga

SEQ ID NO: 15 - DNA, 862 bp, Artificial Sequence
  IMM47C's light chain
atggattcacaggcccaggttcttatgttactgctgctatgggtatctggtacctgtggggacattgtgatgtcacagtctccatcctccctagctgtgtcagttggagagaaggttactatgagctgcaagtccagtcagagccttttatatagtagcaatcaaaagaactacttggcctggtaccagcagaaaccagggcactctcctaaactgctgatttactgggcatccactagggaatctggggtccctgatcgcttcacaggcagtggatctgggacagatttcactctcaccatcagcagtgtgaaggctgaagacctggcagtttattactgtcagcaaaattttatctatccgctcacgttcggtgctgggaccaagctggagctgaaacgtgagttctagaggatccatctgggataagcatgctgttttctgtctgtccctaacatgccctgtgattatccgcaaacaacacacccaagggcagaactttgttacttaaacaccatcctgtttgcttctttcctcaggaactgtggctgcaccatctgtcttcatcttcccgccatctgatgagcagttgaaatctggaactgcctctgttgtgtgcctgctgaataacttctatcccagagaggccaaagtacagtggaaggtggataacgccctccaatcgggtaactcccaggagagtgtcacagagcaggacagcaaggacagcacctacagcctcagcagcaccctgacgctgagcaaagcagactacgagaaacacaaagtctacgcctgcgaagtcacccatcagggcctgagctcgcccgtcacaaagagcttcaacaggggagagtgttag

SEQ ID NO: 16 - DNA, 859 bp, Artificial Sequence
  IMM47's light chain
atgggatggtcatgtatcatcctttttctggtagcaactgcaactggagtacattcagacattcagatgacacagagccctagcagcctgagcgcctccgtgggcgacagagtgaccatcacctgcaagagcagccaaagcctgctgtacagcagcaatcagaagaactacctggcctggtatcagcagaagcctggcaaggcccctaagctgctgatctactgggcctccacaagagagagcggcgtgcctagcagattcagcggcagcggcagcggcaccgacttcaccctgaccatcagcagcctgcagcctgaggacttcgccacctactactgtcagcagaacttcatctaccctctgaccttcggcggaggcaccaaggtggagctgaagcgtgagttctagaggatccatctgggataagcatgctgttttctgtctgtccctaacatgccctgtgattatccgcaaacaacacacccaagggcagaactttgttacttaaacaccatcctgtttgcttctttcctcaggaactgtggctgcaccatctgtcttcatcttcccgccatctgatgagcagttgaaatctggaactgcctctgttgtgtgcctgctgaataacttctatcccagagaggccaaagtacagtggaaggtggataacgccctccaatcgggtaactcccaggagagtgtcacagagcaggacagcaaggacagcacctacagcctcagcagcaccctgacgctgagcaaagcagactacgagaaacacaaagtctacgcctgcgaagtcacccatcagggcctgagctcgcccgtcacaaagagcttcaacaggggagagtgttag

SEQ ID NO: 17 - DNA, 1401 bp, Artificial Sequence
  IMM47H's heavy chain
atgggatggtcatgtatcatcctttttctggtagcaactgcaactggagtacattcagacgtgcagctgcaagagagcggccctggcctggtgaagcctagcgagaccctgagcctgacctgcaccgtgtccggctacagcatcacaagcggctacagctggcactggatcagacagcctcctggcaagggcctggagtggatcggctacatccactacagcggcagcaccaagtacaaccctagcctgaagagcagagtgaccatcagcgtggacacaagcaagaatcagttcagcctgaagctgagcagcgtgaccgccgccgacaccgccgtgtactactgcgctagaggcgccgactacgccctggactactggggacagagaacaagcgtgaccgtgagcagcgctagcaccaagggcccatcggtcttccccctggcaccctcctccaagagcacctctgggggcacagcggccctgggctgcctggtcaaggactacttccccgaaccggtgacggtgtcgtggaactcaggcgccctgaccagcggcgtgcacaccttcccggctgtcctacagtcctcaggactctactccctcagcagcgtggtgaccgtgccctccagcagcttgggcacccagacctacatctgcaacgtgaatcacaagcccagcaacaccaaggtggacaagagagttgagcccaaatcttgtgacaaaactcacacatgcccaccgtgcccagcacctgaactcctggggggaccgtcagtcttcctcttccccccaaaacccaaggacaccctcatgatctcccggacccctgaggtcacatgcgtggtggtggacgtgagccacgaagaccctgaggtcaagttcaactggtatgtggacggcgtggaggtgcataatgccaagacaaagccgcgggaggagcagtacaacgccacgtaccgtgtggtcagcgtcctcaccgtcctgcaccaagactggctgaatggcaaggagtacaagtgcaaggtctccaacaaagccctcccagcccccatcgccgcaaccatctccaaagccaaagggcagccccgagaaccacaggtgtacaccctgcccccatcccgggaggagatgaccaagaaccaagtcagcctgacctgcctggtcaaaggcttctatcccagcgacatcgccgtggagtgggagagcaatgggcagccggagaacaactacaagaccacgcctcccgtgctggactccgacggctccttcttcctctattccaagctcaccgtggacaagagcaggtggcagcaggggaacgtcttctcatgctccgtgatgcatgaggctctgcacaaccactacacgcagaagagcctctccctgtctccgggcaaatga

SEQ ID NO: 18 - DNA, 859 bp, Artificial Sequence
  IMM47H's light chain
atgggatggtcatgtatcatcctttttctggtagcaactgcaactggagtacattcagacatcgtgatgacacagagccctgacagcctggccgtgagcctgggcgagagagccaccatcaactgcaagagctctcagagcctgctgtacagcagcaatcagaagaactacctggcctggtatcagcagaagcctggacagcctcctaagctgctgatctactgggcaagcacaagagagagcggcgtgcctgacagattcagcggcagcggcagcggcaccgacttcaccctgaccatcagcagcctgcaagccgaggacgtggccgtgtactactgtcagcagaacttcatctaccctctgaccttcggcggcggcaccaaggtggagctgaagcgtgagttctagaggatccatctgggataagcatgctgttttctgtctgtccctaacatgccctgtgattatccgcaaacaacacacccaagggcagaactttgttacttaaacaccatcctgtttgcttctttcctcaggaactgtggctgcaccatctgtcttcatcttcccgccatctgatgagcagttgaaatctggaactgcctctgttgtgtgcctgctgaataacttctatcccagagaggccaaagtacagtggaaggtggataacgccctccaatcgggtaactcccaggagagtgtcacagagcaggacagcaaggacagcacctacagcctcagcagcaccctgacgctgagcaaagcagactacgagaaacacaaagtctacgcctgcgaagtcacccatcagggcctgagctcgcccgtcacaaagagcttcaacaggggagagtgttag

SEQ ID NO: 19 - protein, 364 aa, Artificial Sequence
  SIRPalphaD1 mutant-Fc (IMM01)
EEELQVIQPDKSVSVAAGESAILHCTVTSLIPVGPIQWFRGAGPARELIYNQKEGHFPRVTTVSESTKRENMDFSISISAITPADAGTYYCVKFRKGSPDTEFKSGAGTELSVRAKPSAPVVSGPAARATPQHEPKSCDKTHTCPPCPAPELLGGPSVFLFPPKPKDTLMISRTPEVTCVVVDVSHEDPEVKFNWYVDGVEVHNAKTKPREEQYNSTYRVVSVLTVLHQDWLNGKEYKCKVSNKALPAPIEKTISKAKGQPREPQVYTLPPSRDELTKNQVSLTCLVKGFYPSDIAVEWESNGQPENNYKTTPPVLDSDGSFFLYSKLTVDKSRWQQGNVFSCSVMHEALHNHYTQKSLSLSPG

SEQ ID NO: 20 - DNA, 1095 bp, Artificial Sequence
  SIRPalphaD1 mutant-Fc (IMM01)
gaggaggagctgcaggtgattcagcctgacaagtccgtatcagttgcagctggagagtcggccattctgcactgcactgtgacctccctgatccctgtggggcccatccagtggttcagaggagctggaccagcccgggaattaatctacaatcaaaaagaaggccacttcccccgggtaacaactgtttcagagtccacaaagagagaaaacatggacttttccatcagcatcagtgccatcaccccagcagatgccggcacctactactgtgtgaagttccggaaagggagccctgacacggagtttaagtctggagcaggcactgagctgtctgtgcgtgccaaaccctctgcccccgtggtatcgggccctgcggcgagggccacacctcagcacgagcccaaatcttgtgacaaaactcacacatgcccaccgtgcccagcacctgaactcctggggggaccgtcagtcttcctcttccccccaaaacccaaggacaccctcatgatctcccggacccctgaggtcacatgcgtggtggtggacgtgagccacgaagaccctgaggtcaagttcaactggtacgtggacggcgtggaggtgcataatgccaagacaaagccgcgggaggagcagtacaacagcacgtaccgtgtggtcagcgtcctcaccgtcctgcaccaggactggctgaatggcaaggagtacaagtgcaaggtctccaacaaagccctcccagcccccatcgagaaaaccatctccaaagccaaagggcagccccgagaaccacaggtgtacaccctgcccccatcccgggatgagctgaccaagaaccaggtcagcctgacctgcctggtcaaaggcttctatcccagcgacatcgccgtggagtgggagagcaatgggcagccggagaacaactacaagaccacgcctcccgtgctggactccgacggctccttcttcctctacagcaagctcaccgtggacaagagcaggtggcagcaggggaacgtcttctcatgctccgtgatgcatgaggctctgcacaaccactacacgcagaagagcctctccctgtctccgggttga

SEQ ID NO: 21 - DNA, 57 bp, Artificial Sequence
  Nucleotides coding for murine IgG1 heavy chain signal peptide
atgggatggtcatgtatcatcctttttctggtagcaactgcaactggagtacattca

SEQ ID NO: 22 - DNA, 9 bp, Artificial Sequence
  Kozak
gccgccacc